European Patent Application EP 4 613 764 A1, published September 10, 2025. Title: RECOMBINANT TYPE XVII COLLAGEN WITH TRIPLE HELICAL STRUCTURE AND USE THEREOF. Applicant: SHENZHEN LIYING BIOTECHNOLOGY CO., LTD. Application CN. The sequence listing filed with the application follows.

SEQUENCE LISTING (7 sequences)

SEQ ID NO: 1 - protein, 42 aa, synthetic construct
GEKGERGAAGEPGQKGEMGTPGPKGDRGPRGHKGEKGDKGDQ

SEQ ID NO: 2 - protein, 126 aa, synthetic construct
GEKGERGAAGEPGQKGEMGTPGPKGDRGPRGHKGEKGDKGDQGEKGERGAAGEPGQKGEMGTPGPKGDRGPRGHKGEKGDKGDQGEKGERGAAGEPGQKGEMGTPGPKGDRGPRGHKGEKGDKGDQ

SEQ ID NO: 3 - protein, 168 aa, synthetic construct
GEKGERGAAGEPGQKGEMGTPGPKGDRGPRGHKGEKGDKGDQGEKGERGAAGEPGQKGEMGTPGPKGDRGPRGHKGEKGDKGDQGEKGERGAAGEPGQKGEMGTPGPKGDRGPRGHKGEKGDKGDQGEKGERGAAGEPGQKGEMGTPGPKGDRGPRGHKGEKGDKGDQ

SEQ ID NO: 4 - protein, 210 aa, synthetic construct
GEKGERGAAGEPGQKGEMGTPGPKGDRGPRGHKGEKGDKGDQGEKGERGAAGEPGQKGEMGTPGPKGDRGPRGHKGEKGDKGDQGEKGERGAAGEPGQKGEMGTPGPKGDRGPRGHKGEKGDKGDQGEKGERGAAGEPGQKGEMGTPGPKGDRGPRGHKGEKGDKGDQGEKGERGAAGEPGQKGEMGTPGPKGDRGPRGHKGEKGDKGDQ

SEQ ID NO: 5 - protein, 252 aa, synthetic construct
GEKGERGAAGEPGQKGEMGTPGPKGDRGPRGHKGEKGDKGDQGEKGERGAAGEPGQKGEMGTPGPKGDRGPRGHKGEKGDKGDQGEKGERGAAGEPGQKGEMGTPGPKGDRGPRGHKGEKGDKGDQGEKGERGAAGEPGQKGEMGTPGPKGDRGPRGHKGEKGDKGDQGEKGERGAAGEPGQKGEMGTPGPKGDRGPRGHKGEKGDKGDQGEKGERGAAGEPGQKGEMGTPGPKGDRGPRGHKGEKGDKGDQ

SEQ ID NO: 6 - protein, 294 aa, synthetic construct
GEKGERGAAGEPGQKGEMGTPGPKGDRGPRGHKGEKGDKGDQGEKGERGAAGEPGQKGEMGTPGPKGDRGPRGHKGEKGDKGDQGEKGERGAAGEPGQKGEMGTPGPKGDRGPRGHKGEKGDKGDQGEKGERGAAGEPGQKGEMGTPGPKGDRGPRGHKGEKGDKGDQGEKGERGAAGEPGQKGEMGTPGPKGDRGPRGHKGEKGDKGDQGEKGERGAAGEPGQKGEMGTPGPKGDRGPRGHKGEKGDKGDQGEKGERGAAGEPGQKGEMGTPGPKGDRGPRGHKGEKGDKGDQ

SEQ ID NO: 7 - protein, 336 aa, synthetic construct
GEKGERGAAGEPGQKGEMGTPGPKGDRGPRGHKGEKGDKGDQGEKGERGAAGEPGQKGEMGTPGPKGDRGPRGHKGEKGDKGDQGEKGERGAAGEPGQKGEMGTPGPKGDRGPRGHKGEKGDKGDQGEKGERGAAGEPGQKGEMGTPGPKGDRGPRGHKGEKGDKGDQGEKGERGAAGEPGQKGEMGTPGPKGDRGPRGHKGEKGDKGDQGEKGERGAAGEPGQKGEMGTPGPKGDRGPRGHKGEKGDKGDQGEKGERGAAGEPGQKGEMGTPGPKGDRGPRGHKGEKGDKGDQGEKGERGAAGEPGQKGEMGTPGPKGDRGPRGHKGEKGDKGDQ